European Patent Application EP 4 501 955 A1, published February 5, 2025. Title: Polypeptid für eine Tinte für den 3D-Druck. Applicant: Cellbricks GmbH. Application DE. The sequence listing filed with the application follows.

SEQUENCE LISTING (8 sequences)

SEQ ID NO: 1 - protein, 743 aa, synthetic construct
  source 1..743: organism (original language) = Synthetisches Konstrukt
MRFPSIFTAVLFAASSALAAPVNTTTEDETAQIPAEAVIGYSDLEGDFDVAVLPFSNSTNNGLLFINTTIASIAAKEEGVSLEKREAEAEFTGSPGSPGPDGKTGPPGPAGQDGRPGPPGPPGARGQAGPPGFPGPKGAAGEPGKAGERGVPGPPGAVGPAGKDGEAGAQGPPGPAGPAGERGEQGPAGSPGFQGLPGPAGPPGEAGKPGEQGVPGDLGAPGPSGARGERGFPGERGVQGPPGPAGPRGANGAPGNDGAKGDAGAPGAPGSQGAPGLQGMPGERGAAGLPGPKGDRGDAGPKGADGSPGKDGVRGLTGPIGPPGPAGAPGDKGESGPSGPAGPTGARGAPGDRGEPGPPGPAGFAGPPGADGQPGAKGEPGDAGAKGDAGPPGPAGPAGPPGPIGNVGAPGAKGARGSAGPPGATGFPGAAGRVGPPGPSGNAGPPGPPGPAGKEGGKGPRGETGPAGRPGEVGPPGPPGPAGEKGSPGADGPAGAPGTPGPQGIAGQRGVVGLPGQRGERGFPGLPGPSGEPGKQGPSGASGERGPPGPMGPPGLAGPPGESGREGAPGAEGSPGRDGSPGAKGDRGETGPAGPPGAPGAPGAPGPVGPAGKSGDRGETGPAGPTGPVGPVGARGPAGPQGPRGDKGETGEQGDRGIKGHRGFSGLQGPPGPPGSPGEQGPSGASGPAGPRGPPGSAGAPGKDGLNGLPGPIGPPGPRGRTGDAGPVGPPGPPGPPGPPGPP

SEQ ID NO: 2 - protein, 654 aa, synthetic construct
  source 1..654: organism (original language) = Synthetisches Konstrukt
EFTGSPGSPGPDGKTGPPGPAGQDGRPGPPGPPGARGQAGPPGFPGPKGAAGEPGKAGERGVPGPPGAVGPAGKDGEAGAQGPPGPAGPAGERGEQGPAGSPGFQGLPGPAGPPGEAGKPGEQGVPGDLGAPGPSGARGERGFPGERGVQGPPGPAGPRGANGAPGNDGAKGDAGAPGAPGSQGAPGLQGMPGERGAAGLPGPKGDRGDAGPKGADGSPGKDGVRGLTGPIGPPGPAGAPGDKGESGPSGPAGPTGARGAPGDRGEPGPPGPAGFAGPPGADGQPGAKGEPGDAGAKGDAGPPGPAGPAGPPGPIGNVGAPGAKGARGSAGPPGATGFPGAAGRVGPPGPSGNAGPPGPPGPAGKEGGKGPRGETGPAGRPGEVGPPGPPGPAGEKGSPGADGPAGAPGTPGPQGIAGQRGVVGLPGQRGERGFPGLPGPSGEPGKQGPSGASGERGPPGPMGPPGLAGPPGESGREGAPGAEGSPGRDGSPGAKGDRGETGPAGPPGAPGAPGAPGPVGPAGKSGDRGETGPAGPTGPVGPVGARGPAGPQGPRGDKGETGEQGDRGIKGHRGFSGLQGPPGPPGSPGEQGPSGASGPAGPRGPPGSAGAPGKDGLNGLPGPIGPPGPRGRTGDAGPVGPPGPPGPPGPPGPP

SEQ ID NO: 3 - protein, 749 aa, synthetic construct
  source 1..749: organism (original language) = Synthetisches Konstrukt
MRFPSIFTAVLFAASSALAAPVNTTTEDETAQIPAEAVIGYSDLEGDFDVAVLPFSNSTNNGLLFINTTIASIAAKEEGVSLEKREAEAEFTGSPGSPGPDGKTGPPGPAGQDGRPGPPGPPGARGQAGPPGFPGPKGAAGEPGKAGERGVPGPPGAVGPAGKDGEAGAQGPPGPAGPAGERGEQGPAGSPGFQGLPGPAGPPGEAGKPGEQGVPGDLGAPGPSGARGERGFPGERGVQGPPGPAGPRGANGAPGNDGAKGDAGAPGAPGSQGAPGLQGMPGERGAAGLPGPKGDRGDAGPKGADGSPGKDGVRGLTGPIGPPGPAGAPGDKGESGPSGPAGPTGARGAPGDRGEPGPPGPAGFAGPPGADGQPGAKGEPGDAGAKGDAGPPGPAGPAGPPGPIGNVGAPGAKGARGSAGPPGATGFPGAAGRVGPPGPSGNAGPPGPPGPAGKEGGKGPRGETGPAGRPGEVGPPGPPGPAGEKGSPGADGPAGAPGTPGPQGIAGQRGVVGLPGQRGERGFPGLPGPSGEPGKQGPSGASGERGPPGPMGPPGLAGPPGESGREGAPGAEGSPGRDGSPGAKGDRGETGPAGPPGAPGAPGAPGPVGPAGKSGDRGETGPAGPTGPVGPVGARGPAGPQGPRGDKGETGEQGDRGIKGHRGFSGLQGPPGPPGSPGEQGPSGASGPAGPRGPPGSAGAPGKDGLNGLPGPIGPPGPRGRTGDAGPVGPPGPPGPPGPPGPPHHHHHH

SEQ ID NO: 4 - protein, 660 aa, synthetic construct
  source 1..660: organism (original language) = Synthetisches Konstrukt
EFTGSPGSPGPDGKTGPPGPAGQDGRPGPPGPPGARGQAGPPGFPGPKGAAGEPGKAGERGVPGPPGAVGPAGKDGEAGAQGPPGPAGPAGERGEQGPAGSPGFQGLPGPAGPPGEAGKPGEQGVPGDLGAPGPSGARGERGFPGERGVQGPPGPAGPRGANGAPGNDGAKGDAGAPGAPGSQGAPGLQGMPGERGAAGLPGPKGDRGDAGPKGADGSPGKDGVRGLTGPIGPPGPAGAPGDKGESGPSGPAGPTGARGAPGDRGEPGPPGPAGFAGPPGADGQPGAKGEPGDAGAKGDAGPPGPAGPAGPPGPIGNVGAPGAKGARGSAGPPGATGFPGAAGRVGPPGPSGNAGPPGPPGPAGKEGGKGPRGETGPAGRPGEVGPPGPPGPAGEKGSPGADGPAGAPGTPGPQGIAGQRGVVGLPGQRGERGFPGLPGPSGEPGKQGPSGASGERGPPGPMGPPGLAGPPGESGREGAPGAEGSPGRDGSPGAKGDRGETGPAGPPGAPGAPGAPGPVGPAGKSGDRGETGPAGPTGPVGPVGARGPAGPQGPRGDKGETGEQGDRGIKGHRGFSGLQGPPGPPGSPGEQGPSGASGPAGPRGPPGSAGAPGKDGLNGLPGPIGPPGPRGRTGDAGPVGPPGPPGPPGPPGPPHHHHHH

SEQ ID NO: 5 - DNA, 2232 bp, synthetic construct
  source 1..2232: mol_type = other DNA; organism (original language) = Synthetisches Konstrukt
atgagatttccttcaatttttactgcagttttattcgcagcatcctccgcattagctgctccagtcaacactacaacagaagatgaaacggcacaaattccggctgaagctgtcatcggttactcagatttagaaggggatttcgatgttgctgttttgccattttccaacagcacaaataacgggttattgtttataaatactactattgccagcattgctgctaaagaagaaggggtatctctcgagaaaagagaggctgaagctgaattcactggttccccaggttctccaggtccagatggtaaaactggtccaccaggtcctgctggacaagatggtagaccaggtccacctggaccacctggtgctagaggtcaagctggtcctcctggttttcctggtccaaaaggtgcagctggtgaaccaggtaaggctggtgaaagaggtgttccaggacctccaggtgctgttggacctgctggtaaagacggtgaagctggtgctcaaggtcctccaggaccagccggaccagcaggcgagagaggtgaacaaggacctgcaggatctccaggatttcaaggtttacccggtccagctggcccaccaggcgaagctggtaaacctggtgagcaaggtgttcctggtgatttgggtgctcctggtccttcaggtgcaagaggtgaaaggggtttcccaggtgaacgtggtgtacagggacctcctggacctgccggtcctagaggtgctaatggtgctccaggtaatgatggtgctaagggtgatgccggcgctcctggtgcacctggatctcaaggtgccccaggtctacaaggtatgcccggtgagaggggtgctgctggtttgccaggacctaaaggtgatagaggtgatgctggaccaaagggtgctgatggatcacctggtaaggatggtgttagaggtttgactggtccaatcggaccaccaggtccagccggtgctcccggtgataagggcgaatctggaccctctggtcctgccggaccaactggcgctaggggtgcccctggtgatcgtggtgagcctggacctccaggtcctgccggatttgctggtccacctggtgcagatggacaaccaggtgctaaaggcgaaccaggtgacgccggtgccaaaggtgacgcaggcccacctggtcctgcaggccccgctggaccaccaggacctattggtaatgttggagccccaggtgccaagggtgccagaggatcagcaggccctccaggcgctactggtttccctggcgctgctggtagagttggccctcctggtccatctggtaatgctggccctccaggacctcctggtccagccggcaaagaaggtggtaaaggaccaaggggtgaaactggcccagctggtaggccaggtgaggtaggaccacctggtcctccaggtccagctggtgaaaaaggttctcctggtgctgacggtcccgctggcgctcccggtactcccggaccacaaggtattgcaggtcagagaggtgttgttggattgcctggacaaagaggtgagagaggatttcctggattgccaggtccatcaggcgaacctggaaagcaaggacctagtggtgcatctggcgaaagaggcccaccaggaccaatgggtcctcctggattagcaggtcctcctggcgaatctggtagagaaggtgctccaggcgctgaaggatctcctggtagagatggatctcccggtgcaaaaggcgatagaggcgaaactggtcccgctggacctcctggcgctccaggtgctcctggtgctcccggtcctgtcggtcctgctggaaaatctggtgacagaggtgaaaccggacctgctggcccaactggtccagtcggtccagttggagctagaggacccgcaggacctcagggtcccagaggcgataagggtgagactggtgaacagggtgaccgtggtattaagggtcacagaggtttttctggtctgcagggcccaccaggtcctccaggatctccaggtgaacaaggtccttctggtgcttctggaccagctggccctcgtggcccacctggatctgctggtgctcctggaaaagatggtttgaacggtttgcctggtcctataggtcctcctggtcctagaggtagaactggtgatgccggtcctgtgggacctccaggtccacctggtcctccaggacctcctggaccaccataa

SEQ ID NO: 6 - DNA, 1965 bp, synthetic construct
  source 1..1965: mol_type = other DNA; organism (original language) = Synthetisches Konstrukt
gaattcactggttccccaggttctccaggtccagatggtaaaactggtccaccaggtcctgctggacaagatggtagaccaggtccacctggaccacctggtgctagaggtcaagctggtcctcctggttttcctggtccaaaaggtgcagctggtgaaccaggtaaggctggtgaaagaggtgttccaggacctccaggtgctgttggacctgctggtaaagacggtgaagctggtgctcaaggtcctccaggaccagccggaccagcaggcgagagaggtgaacaaggacctgcaggatctccaggatttcaaggtttacccggtccagctggcccaccaggcgaagctggtaaacctggtgagcaaggtgttcctggtgatttgggtgctcctggtccttcaggtgcaagaggtgaaaggggtttcccaggtgaacgtggtgtacagggacctcctggacctgccggtcctagaggtgctaatggtgctccaggtaatgatggtgctaagggtgatgccggcgctcctggtgcacctggatctcaaggtgccccaggtctacaaggtatgcccggtgagaggggtgctgctggtttgccaggacctaaaggtgatagaggtgatgctggaccaaagggtgctgatggatcacctggtaaggatggtgttagaggtttgactggtccaatcggaccaccaggtccagccggtgctcccggtgataagggcgaatctggaccctctggtcctgccggaccaactggcgctaggggtgcccctggtgatcgtggtgagcctggacctccaggtcctgccggatttgctggtccacctggtgcagatggacaaccaggtgctaaaggcgaaccaggtgacgccggtgccaaaggtgacgcaggcccacctggtcctgcaggccccgctggaccaccaggacctattggtaatgttggagccccaggtgccaagggtgccagaggatcagcaggccctccaggcgctactggtttccctggcgctgctggtagagttggccctcctggtccatctggtaatgctggccctccaggacctcctggtccagccggcaaagaaggtggtaaaggaccaaggggtgaaactggcccagctggtaggccaggtgaggtaggaccacctggtcctccaggtccagctggtgaaaaaggttctcctggtgctgacggtcccgctggcgctcccggtactcccggaccacaaggtattgcaggtcagagaggtgttgttggattgcctggacaaagaggtgagagaggatttcctggattgccaggtccatcaggcgaacctggaaagcaaggacctagtggtgcatctggcgaaagaggcccaccaggaccaatgggtcctcctggattagcaggtcctcctggcgaatctggtagagaaggtgctccaggcgctgaaggatctcctggtagagatggatctcccggtgcaaaaggcgatagaggcgaaactggtcccgctggacctcctggcgctccaggtgctcctggtgctcccggtcctgtcggtcctgctggaaaatctggtgacagaggtgaaaccggacctgctggcccaactggtccagtcggtccagttggagctagaggacccgcaggacctcagggtcccagaggcgataagggtgagactggtgaacagggtgaccgtggtattaagggtcacagaggtttttctggtctgcagggcccaccaggtcctccaggatctccaggtgaacaaggtccttctggtgcttctggaccagctggccctcgtggcccacctggatctgctggtgctcctggaaaagatggtttgaacggtttgcctggtcctataggtcctcctggtcctagaggtagaactggtgatgccggtcctgtgggacctccaggtccacctggtcctccaggacctcctggaccaccataa

SEQ ID NO: 7 - DNA, 2250 bp, synthetic construct
  source 1..2250: mol_type = other DNA; organism (original language) = Synthetisches Konstrukt
atgagatttccttcaatttttactgcagttttattcgcagcatcctccgcattagctgctccagtcaacactacaacagaagatgaaacggcacaaattccggctgaagctgtcatcggttactcagatttagaaggggatttcgatgttgctgttttgccattttccaacagcacaaataacgggttattgtttataaatactactattgccagcattgctgctaaagaagaaggggtatctctcgagaaaagagaggctgaagctgaattcactggttccccaggttctccaggtccagatggtaaaactggtccaccaggtcctgctggacaagatggtagaccaggtccacctggaccacctggtgctagaggtcaagctggtcctcctggttttcctggtccaaaaggtgcagctggtgaaccaggtaaggctggtgaaagaggtgttccaggacctccaggtgctgttggacctgctggtaaagacggtgaagctggtgctcaaggtcctccaggaccagccggaccagcaggcgagagaggtgaacaaggacctgcaggatctccaggatttcaaggtttacccggtccagctggcccaccaggcgaagctggtaaacctggtgagcaaggtgttcctggtgatttgggtgctcctggtccttcaggtgcaagaggtgaaaggggtttcccaggtgaacgtggtgtacagggacctcctggacctgccggtcctagaggtgctaatggtgctccaggtaatgatggtgctaagggtgatgccggcgctcctggtgcacctggatctcaaggtgccccaggtctacaaggtatgcccggtgagaggggtgctgctggtttgccaggacctaaaggtgatagaggtgatgctggaccaaagggtgctgatggatcacctggtaaggatggtgttagaggtttgactggtccaatcggaccaccaggtccagccggtgctcccggtgataagggcgaatctggaccctctggtcctgccggaccaactggcgctaggggtgcccctggtgatcgtggtgagcctggacctccaggtcctgccggatttgctggtccacctggtgcagatggacaaccaggtgctaaaggcgaaccaggtgacgccggtgccaaaggtgacgcaggcccacctggtcctgcaggccccgctggaccaccaggacctattggtaatgttggagccccaggtgccaagggtgccagaggatcagcaggccctccaggcgctactggtttccctggcgctgctggtagagttggccctcctggtccatctggtaatgctggccctccaggacctcctggtccagccggcaaagaaggtggtaaaggaccaaggggtgaaactggcccagctggtaggccaggtgaggtaggaccacctggtcctccaggtccagctggtgaaaaaggttctcctggtgctgacggtcccgctggcgctcccggtactcccggaccacaaggtattgcaggtcagagaggtgttgttggattgcctggacaaagaggtgagagaggatttcctggattgccaggtccatcaggcgaacctggaaagcaaggacctagtggtgcatctggcgaaagaggcccaccaggaccaatgggtcctcctggattagcaggtcctcctggcgaatctggtagagaaggtgctccaggcgctgaaggatctcctggtagagatggatctcccggtgcaaaaggcgatagaggcgaaactggtcccgctggacctcctggcgctccaggtgctcctggtgctcccggtcctgtcggtcctgctggaaaatctggtgacagaggtgaaaccggacctgctggcccaactggtccagtcggtccagttggagctagaggacccgcaggacctcagggtcccagaggcgataagggtgagactggtgaacagggtgaccgtggtattaagggtcacagaggtttttctggtctgcagggcccaccaggtcctccaggatctccaggtgaacaaggtccttctggtgcttctggaccagctggccctcgtggcccacctggatctgctggtgctcctggaaaagatggtttgaacggtttgcctggtcctataggtcctcctggtcctagaggtagaactggtgatgccggtcctgtgggacctccaggtccacctggtcctccaggacctcctggaccaccacatcaccatcatcatcactaa

SEQ ID NO: 8 - DNA, 1983 bp, synthetic construct
  source 1..1983: mol_type = other DNA; organism (original language) = Synthetisches Konstrukt
gaattcactggttccccaggttctccaggtccagatggtaaaactggtccaccaggtcctgctggacaagatggtagaccaggtccacctggaccacctggtgctagaggtcaagctggtcctcctggttttcctggtccaaaaggtgcagctggtgaaccaggtaaggctggtgaaagaggtgttccaggacctccaggtgctgttggacctgctggtaaagacggtgaagctggtgctcaaggtcctccaggaccagccggaccagcaggcgagagaggtgaacaaggacctgcaggatctccaggatttcaaggtttacccggtccagctggcccaccaggcgaagctggtaaacctggtgagcaaggtgttcctggtgatttgggtgctcctggtccttcaggtgcaagaggtgaaaggggtttcccaggtgaacgtggtgtacagggacctcctggacctgccggtcctagaggtgctaatggtgctccaggtaatgatggtgctaagggtgatgccggcgctcctggtgcacctggatctcaaggtgccccaggtctacaaggtatgcccggtgagaggggtgctgctggtttgccaggacctaaaggtgatagaggtgatgctggaccaaagggtgctgatggatcacctggtaaggatggtgttagaggtttgactggtccaatcggaccaccaggtccagccggtgctcccggtgataagggcgaatctggaccctctggtcctgccggaccaactggcgctaggggtgcccctggtgatcgtggtgagcctggacctccaggtcctgccggatttgctggtccacctggtgcagatggacaaccaggtgctaaaggcgaaccaggtgacgccggtgccaaaggtgacgcaggcccacctggtcctgcaggccccgctggaccaccaggacctattggtaatgttggagccccaggtgccaagggtgccagaggatcagcaggccctccaggcgctactggtttccctggcgctgctggtagagttggccctcctggtccatctggtaatgctggccctccaggacctcctggtccagccggcaaagaaggtggtaaaggaccaaggggtgaaactggcccagctggtaggccaggtgaggtaggaccacctggtcctccaggtccagctggtgaaaaaggttctcctggtgctgacggtcccgctggcgctcccggtactcccggaccacaaggtattgcaggtcagagaggtgttgttggattgcctggacaaagaggtgagagaggatttcctggattgccaggtccatcaggcgaacctggaaagcaaggacctagtggtgcatctggcgaaagaggcccaccaggaccaatgggtcctcctggattagcaggtcctcctggcgaatctggtagagaaggtgctccaggcgctgaaggatctcctggtagagatggatctcccggtgcaaaaggcgatagaggcgaaactggtcccgctggacctcctggcgctccaggtgctcctggtgctcccggtcctgtcggtcctgctggaaaatctggtgacagaggtgaaaccggacctgctggcccaactggtccagtcggtccagttggagctagaggacccgcaggacctcagggtcccagaggcgataagggtgagactggtgaacagggtgaccgtggtattaagggtcacagaggtttttctggtctgcagggcccaccaggtcctccaggatctccaggtgaacaaggtccttctggtgcttctggaccagctggccctcgtggcccacctggatctgctggtgctcctggaaaagatggtttgaacggtttgcctggtcctataggtcctcctggtcctagaggtagaactggtgatgccggtcctgtgggacctccaggtccacctggtcctccaggacctcctggaccaccacatcaccatcatcatcactaa